European Patent Specification EP 3 521 308 B1, published March 13, 2024. Title: Humanized and de-immunized antibodies. Applicant: Probiodrug AG. The sequence listing filed with the application follows.

SEQUENCE LISTING (49 sequences)

SEQ ID NO: 1 - protein, 112 aa, Artificial sequence
  Recombinant Polypeptide
DVVMTQSPLSLPVTLGQPASISCKSSQSLLYSDGKTYLNWFQQRPGQSPRRLTYLVSKLDSGVPDRFSGSGSGTDFTLKISRVEAEDVGVYYCVQGTHFPFTFGGGTKVEIK

SEQ ID NO: 2 - protein, 119 aa, Artificial sequence
  Recombinant Polypeptide
QVQLVQSGAEVVKPGASVKVSCKASGYSFTGHTMNWVRQAPGQGLEWMGLINPSDGVTRYNQKFQGRVTITRDTSTTTVHMELTSLTSEDTATYYCTREAKREWDETYWGQGTLVTVSS

SEQ ID NO: 3 - protein, 15 aa, Artificial sequence
  Recombinant peptide
SSQSLLYSDGKTYLN

SEQ ID NO: 4 - protein, 7 aa, Artificial sequence
  Synthetic peptide
LVSKLDS

SEQ ID NO: 5 - protein, 7 aa, Artificial sequence
  Recombinant peptide
VQGTHFP

SEQ ID NO: 6 - protein, 10 aa, Artificial sequence
  Recombinant peptide
GYSFTGHTMN

SEQ ID NO: 7 - protein, 17 aa, Artificial sequence
  Recombinant peptide
LINPSDGVTRYNQKFQG

SEQ ID NO: 8 - protein, 10 aa, Artificial sequence
  Recombinant peptide
EAKREWDETY

SEQ ID NO: 9 - DNA, 336 bp, Artificial sequence
  Recombinant nucleic acid
gacgtggtgatgactcagtctccactctccctgcccgtcacccttggacagccggcctccatctcctgcaagtcaagtcagagcctcctgcactccgacggcaagacctacttgaactggttccagcagaggccaggccagtctccaaggcgcctgacctatctggtgtctaagctggactctggggtcccagacagattcagcggcagtgggtcaggcactgacttcacactgaagatcagcagggtggaggctgaggatgtcggagtctactactgcgtgcaaggtacacacttcccattcacgttcggcggagggaccaaggtggaaatcaaa

SEQ ID NO: 10 - DNA, 357 bp, Artificial sequence
  Synthetic nucleic acid
caggtgcagctcgtgcagtctggggctgaggtggtgaagccaggtgcctcagtgaaggtctcctgcaaggcatctggttactcattcactggtcacaccatgaactgggtgcgacaggcccctggacaagggcttgagtggatgggactcatcaatccttccgatggtgttactaggtacaaccagaagttccagggcagagtcaccatcaccagggacacgtccacgaccaccgttcacatggagctgaccagcctgacatctgaggacacggccacctactactgtacgagagaggcgaaacgggagtgggacgagacttactggggccagggaaccctggtcaccgtctcctca

SEQ ID NO: 11 - DNA, 45 bp, Artificial sequence
  Recombinant nucleic acid
tcaagtcagagcctcctgcactccgacggcaagacctacttgaac

SEQ ID NO: 12 - DNA, 21 bp, Artificial sequence
  Recombinant nucleic acid
ctggtgtctaagctggactct

SEQ ID NO: 13 - DNA, 21 bp, Artificial sequence
  Recombinant nucleic acid
gtgcaaggtacacacttccca

SEQ ID NO: 14 - DNA, 30 bp, Artificial sequence
  Recombinant nucleic acid
ggttactcattcactggtcacaccatgaac

SEQ ID NO: 15 - DNA, 51 bp, Artificial sequence
  Recombinant nucleic acid
ctcatcaatccttccgatggtgttactaggtacaaccagaagttccagggc

SEQ ID NO: 16 - DNA, 30 bp, Artificial sequence
  Recombinant nucleic acid
gaggcgaaacgggagtgggacgagacttac

SEQ ID NO: 17 - protein, 219 aa, Artificial sequence
  Recombinant polypeptide
DVVMTQSPLSLPVTLGQPASISCKSSQSLLYSDGKTYLNWFQQRPGQSPRRLTYLVSKLDSGVPDRFSGSGSGTDFTLKISRVEAEDVGVYYCVQGTHFPFTFGGGTKVEIKRTVAAPSVFIFPPSDEQLKSGTASVVCLLNNFYPREAKVQWKVDNALQSGNSQESVTEQDSKDSTYSLSSTLTLSKADYEKHKVYACEVTHQGLSSPVTKSFNRGEC

SEQ ID NO: 18 - protein, 449 aa, Artificial sequence
  Recombinant polypeptide
QVQLVQSGAEVVKPGASVKVSCKASGYSFTGHTMNWVRQAPGQGLEWMGLINPSDGVTRYNQKFQGRVTITRDTSTTTVHMELTSLTSEDTATYYCTREAKREWDETYWGQGTLVTVSSASTKGPSVFPLAPSSKSTSGGTAALGCLVKDYFPEPVTVSWNSGALTSGVHTFPAVLQSSGLYSLSSVVTVPSSSLGTQTYICNVNHKPSNTKVDKKVEPKSCDKTHTCPPCPAPELLGGPSVFLFPPKPKDTLMISRTPEVTCVVVDVSHEDPEVKFNWYVDGVEVHNAKTKPREEQYNSTYRVVSVLTVLHQDWLNGKEYKCAVSNKALPAPIEKTISKAKGQPREPQVYTLPPSRDELTKNQVSLTCLVKGFYPSDIAVEWESNGQPENNYKTTPPVLDSDGSFFLYSKLTVDKSRWQQGNVFSCSVMHEALHNHYTQKSLSLSPGK

SEQ ID NO: 19 - protein, 449 aa, Artificial sequence
  Recombinant polypeptide
QVQLVQSGAEVVKPGASVKVSCKASGYSFTGHTMNWVRQAPGQGLEWMGLINPSDGVTRYNQKFQGRVTITRDTSTTTVHMELTSLTSEDTATYYCTREAKREWDETYWGQGTLVTVSSASTKGPSVFPLAPSSKSTSGGTAALGCLVKDYFPEPVTVSWNSGALTSGVHTFPAVLQSSGLYSLSSVVTVPSSSLGTQTYICNVNHKPSNTKVDKKVEPKSCDKTHTCPPCPAPELLGGPSVFLFPPKPKDTLMISRTPEVTCVVVDVSHEDPEVKFNWYVDGVEVHNAKTKPREEQYNSTYRVVSVLTVLHQDWLNGKEYKCKVSNKALPAPIEKTISKAKGQPREPQVYTLPPSRDELTKNQVSLTCLVKGFYPSDIAVEWESNGQPENNYKTTPPVLDSDGSFFLYSKLTVDKSRWQQGNVFSCSVMHEALHNHYTQKSLSLSPGK

SEQ ID NO: 20 - DNA, 657 bp, Artificial sequence
  Recombinant nucleic acid
gacgtggtgatgactcagtctccactctccctgcccgtcacccttggacagccggcctccatctcctgcaagtcaagtcagagcctcctgcactccgacggcaagacctacttgaactggttccagcagaggccaggccagtctccaaggcgcctgacctatctggtgtctaagctggactctggggtcccagacagattcagcggcagtgggtcaggcactgacttcacactgaagatcagcagggtggaggctgaggatgtcggagtctactactgcgtgcaaggtacacacttcccattcacgttcggcggagggaccaaggtggaaatcaaaaggaccgtggccgcaccctctgtgttcatcttcccccccagcgacgagcagctgaagagcggcactgcatctgtcgtgtgtctgctgaacaacttctacccaagggaggcgaaagtgcagtggaaggtagacaacgccttgcaatccggcaactcccaggagagcgtgaccgagcaggacagcaaagactcaacctacagcctgagcagtactttgaccctgtctaaggccgattacgagaagcacaaggtgtacgcctgcgaggtaacccaccagggactgagctctcccgtgaccaagagcttcaacaggggcgagtgc

SEQ ID NO: 21 - DNA, 1347 bp, Artificial sequence
  Recombinant nucleic acid
caggtgcagctcgtgcagtctggggctgaggtggtgaagccaggtgcctcagtgaaggtctcctgcaaggcatctggttactcattcactggtcacaccatgaactgggtgcgacaggcccctggacaagggcttgagtggatgggactcatcaatccttccgatggtgttactaggtacaaccagaagttccagggcagagtcaccatcaccagggacacgtccacgaccaccgttcacatggagctgaccagcctgacatctgaggacacggccacctactactgtacgagagaggcgaaacgggagtgggacgagacttactggggccagggaaccctggtcaccgtctcctcagccagcactaagggcccgagcgtgttccccctcgcccctagcagtaagagcaccagcggtggcacggcggcacttggctgcttggttaaggactacttcccagagcccgtgaccgtgtcctggaactctggggcacttaccagtggcgtgcacaccttccccgctgtactgcagagcagcggcttgtacagcttgtcttccgtcgtaacggtgcccagcagcagcttgggaacccagacctacatctgcaacgtaaaccacaagccatccaacaccaaggtagacaaaaaggtcgaacccaagtcctgcgacaagacccacacctgtccaccctgtcctgcacccgagctcctgggaggtcccagcgttttcctgttccctccaaagccaaaggataccctgatgatcagcaggacccccgaggtgacctgcgtggtggtggacgtgagccacgaagaccctgaggtcaagttcaactggtacgttgatggggtggaggtacacaatgccaagaccaaacctcgagaggagcaatacaacagcacctaccgagttgtgagcgtgcttaccgtgctgcaccaggactggctgaacggcaaggagtacaagtgcgctgtgagcaacaaggctctgccggctcccatcgagaagaccatcagcaaggccaagggccagcccagggagccacaggtttacacgttgcccccctcaagggacgagttgaccaagaaccaggtttccctcacgtgccttgtgaagggcttctaccccagcgacatcgccgtggaatgggagagcaacgggcagcccgagaacaactacaagacgaccccccctgttctggacagcgacggctctttcttcctgtattcaaagctcaccgtggacaaaagcaggtggcagcagggtaatgtgttctcctgcagcgtgatgcacgaggccctgcataaccactacacccaaaagagcttgagcctctcccccggtaag

SEQ ID NO: 22 - DNA, 1347 bp, Artificial sequence
  Recombinant nucleic acid
caggtgcagctcgtgcagtctggggctgaggtggtgaagccaggtgcctcagtgaaggtctcctgcaaggcatctggttactcattcactggtcacaccatgaactgggtgcgacaggcccctggacaagggcttgagtggatgggactcatcaatccttccgatggtgttactaggtacaaccagaagttccagggcagagtcaccatcaccagggacacgtccacgaccaccgttcacatggagctgaccagcctgacatctgaggacacggccacctactactgtacgagagaggcgaaacgggagtgggacgagacttactggggccagggaaccctggtcaccgtctcctcagccagcactaagggcccgagcgtgttccccctcgcccctagcagtaagagcaccagcggtggcacggcggcacttggctgcttggttaaggactacttcccagagcccgtgaccgtgtcctggaactctggggcacttaccagtggcgtgcacaccttccccgctgtactgcagagcagcggcttgtacagcttgtcttccgtcgtaacggtgcccagcagcagcttgggaacccagacctacatctgcaacgtaaaccacaagccatccaacaccaaggtagacaaaaaggtcgaacccaagtcctgcgacaagacccacacctgtccaccctgtcctgcacccgagctcctgggaggtcccagcgttttcctgttccctccaaagccaaaggataccctgatgatcagcaggacccccgaggtgacctgcgtggtggtggacgtgagccacgaagaccctgaggtcaagttcaactggtacgttgatggggtggaggtacacaatgccaagaccaaacctcgagaggagcaatacaacagcacctaccgagttgtgagcgtgcttaccgtgctgcaccaggactggctgaacggcaaggagtacaagtgcaaggtgagcaacaaggctctgccggctcccatcgagaagaccatcagcaaggccaagggccagcccagggagccacaggtttacacgttgcccccctcaagggacgagttgaccaagaaccaggtttccctcacgtgccttgtgaagggcttctaccccagcgacatcgccgtggaatgggagagcaacgggcagcccgagaacaactacaagacgaccccccctgttctggacagcgacggctctttcttcctgtattcaaagctcaccgtggacaaaagcaggtggcagcagggtaatgtgttctcctgcagcgtgatgcacgaggccctgcataaccactacacccaaaagagcttgagcctctcccccggtaag

SEQ ID NO: 23 - protein, 16 aa, Artificial sequence
  Synthetic peptide
  MOD_RES (1)..(1): PYRROLIDONE CARBOXYLIC ACID
EFRHDSGYEVHHQKLV

SEQ ID NO: 24 - protein, 15 aa, Artificial sequence
  Synthetic peptide
  MOD_RES (1)..(1): PYRROLIDONE CARBOXYLIC ACID
EFRHDSGYEVHHQKL

SEQ ID NO: 25 - protein, 14 aa, Artificial sequence
  Synthetic peptide
  MOD_RES (1)..(1): PYRROLIDONE CARBOXYLIC ACID
EFRHDSGYEVHHQK

SEQ ID NO: 26 - protein, 13 aa, Artificial sequence
  Synthetic peptide
  MOD_RES (1)..(1): PYRROLIDONE CARBOXYLIC ACID
EFRHDSGYEVHHQ

SEQ ID NO: 27 - protein, 12 aa, Artificial sequence
  Synthetic peptide
  MOD_RES (1)..(1): PYRROLIDONE CARBOXYLIC ACID
EFRHDSGYEVHH

SEQ ID NO: 28 - protein, 11 aa, Artificial sequence
  Synthetic peptide
  MOD_RES (1)..(1): PYRROLIDONE CARBOXYLIC ACID
EFRHDSGYEVH

SEQ ID NO: 29 - protein, 10 aa, Artificial sequence
  Synthetic peptide
  MOD_RES (1)..(1): PYRROLIDONE CARBOXYLIC ACID
EFRHDSGYEV

SEQ ID NO: 30 - protein, 9 aa, Artificial sequence
  Synthetic peptide
  MOD_RES (1)..(1): PYRROLIDONE CARBOXYLIC ACID
EFRHDSGYE

SEQ ID NO: 31 - protein, 8 aa, Artificial sequence
  Synthetic peptide
  MOD_RES (1)..(1): PYRROLIDONE CARBOXYLIC ACID
EFRHDSGY

SEQ ID NO: 32 - protein, 7 aa, Artificial sequence
  Synthetic peptide
  MOD_RES (1)..(1): PYRROLIDONE CARBOXYLIC ACID
EFRHDSG

SEQ ID NO: 33 - protein, 6 aa, Artificial sequence
  Synthetic peptide
  MOD_RES (1)..(1): PYRROLIDONE CARBOXYLIC ACID
EFRHDS

SEQ ID NO: 34 - protein, 5 aa, Artificial sequence
  Synthetic peptide
  MOD_RES (1)..(1): PYRROLIDONE CARBOXYLIC ACID
EFRHD

SEQ ID NO: 35 - protein, 4 aa, Artificial sequence
  Synthetic peptide
  MOD_RES (1)..(1): PYRROLIDONE CARBOXYLIC ACID
EFRH

SEQ ID NO: 36 - protein, 3 aa, Artificial sequence
  Synthetic peptide
  MOD_RES (1)..(1): PYRROLIDONE CARBOXYLIC ACID
EFR

SEQ ID NO: 37 - protein, 42 aa, Human [sequence omitted]

SEQ ID NO: 38 - protein, 40 aa, Human
DAEFRHDSGYEVHHQKLVFFAEDVGSNKGAIIGLMVGGVV

SEQ ID NO: 39 - protein, 38 aa, Human
DAEFRHDSGYEVHHQKLVFFAEDVGSNKGAIIGLMVGG

SEQ ID NO: 40 - protein, 40 aa, Human
EFRHDSGYEVHHQKLVFFAEDVGSNKGAIIGLMVGGVVIA

SEQ ID NO: 41 - protein, 38 aa, Human
EFRHDSGYEVHHQKLVFFAEDVGSNKGAIIGLMVGGVV

SEQ ID NO: 42 - protein, 36 aa, Human
EFRHDSGYEVHHQKLVFFAEDVGSNKGAIIGLMVGG

SEQ ID NO: 43 - DNA, 24 bp, Artificial sequence
  PCR primer
actgtggctgcaccatctgtcttc

SEQ ID NO: 44 - DNA, 25 bp, Artificial sequence
  PCR primer
ctaacactctcccctgttgaagctc

SEQ ID NO: 45 - DNA, 23 bp, Artificial sequence
  PCR primer
agggaaccctggtcaccgtctcc

SEQ ID NO: 46 - DNA, 25 bp, Artificial sequence
  PCR primer
tcatttacccggagacagggagagg

SEQ ID NO: 47 - DNA, 24 bp, Artificial sequence
  PCR primer
caagtcagagcctcttatatagtg

SEQ ID NO: 48 - DNA, 23 bp, Artificial sequence
  PCR primer
gtaccttgcacgcagtaataaac

SEQ ID NO: 49 - protein, 119 aa, Artificial sequence
  Recombinant polypeptide
QVQLVQSGAEVKKSGASVKVSCKASGYSFTGHTMNWVRQAPGQGLEWMGLINPSNGVTRYNQKFQGRVTITRDTSTTTVHMELTSLTSEDTATYYCTREAKREWDETYWGQGTLVTVSS